European Patent Application EP 4 748 847 A1, published May 27, 2026. Title: ＶＥＧＦＲ－２アゴニスト活性を有するペプチド複合体. Applicant: ペプチドリーム株式会社. The sequence listing filed with the application follows.

SEQUENCE LISTING (51 sequences)

SEQ ID NO: 1 - skipped

SEQ ID NO: 2 - protein, 14 aa, synthetic construct
WWVDVQDDLYFVDC

SEQ ID NO: 3 - protein, 15 aa, synthetic construct
WWVDVQDDLYFVDCG

SEQ ID NO: 4 - protein, 15 aa, synthetic construct
  MOD_RES 6: note = X represents (S)-2-Aminoheptanoic acid(Ahp)
WWVDVXDDLYFVDCG

SEQ ID NO: 5 - protein, 15 aa, synthetic construct
WWVDVWDDLYFVDCG

SEQ ID NO: 6 - protein, 15 aa, synthetic construct
  MOD_RES 6: note = F represents (S)-2-Amino-4-phenylbutanoic acid(Hph)
WWVDVFDDLYFVDCG

SEQ ID NO: 7 - protein, 15 aa, synthetic construct
  MOD_RES 6: note = A represents (S)-2-Amino-3-cyclohexylpropanoic acid(Cha)
WWVDVADDLYFVDCG

SEQ ID NO: 8 - protein, 15 aa, synthetic construct
  MOD_RES 6: note = F represents 4-Carboxy-L-phenylalanine(F4COO)
WWVDVFDDLYFVDCG

SEQ ID NO: 9 - protein, 15 aa, synthetic construct
WWVDVQGDLYFVDCG

SEQ ID NO: 10 - protein, 15 aa, synthetic construct
  MOD_RES 11: note = A represents (S)-3-([1,1'-Biphenyl]-4-yl)-2-aminopropanoic acid(Bph)
WWVDVQDDLYAVDCG

SEQ ID NO: 11 - protein, 15 aa, synthetic construct
  MOD_RES 12: note = F represents (S)-2-Amino-4-phenylbutanoic acid(Hph)
WWVDVQDDLYFFDCG

SEQ ID NO: 12 - protein, 15 aa, synthetic construct
WWVDVQDDLYFVACG

SEQ ID NO: 13 - protein, 15 aa, synthetic construct
WWVDVQDDLYFVSCG

SEQ ID NO: 14 - protein, 15 aa, synthetic construct
WWVDVKDDLYFVDCG

SEQ ID NO: 15 - protein, 15 aa, synthetic construct
  MOD_RES 5: note = L represents (S)-2-Amino-3,3-dimethylbutanoic acid(Tbg)
WWVDLKDDLYFVDCG

SEQ ID NO: 16 - protein, 15 aa, synthetic construct
  MOD_RES 11: note = Y represents (S)-2-Amino-3-(4-phenoxyphenyl)propanoic acid(Yph)
WWVDVKDDLYYVDCG

SEQ ID NO: 17 - protein, 15 aa, synthetic construct
  MOD_RES 11: note = F represents (S)-2-Amino-3-(4-guanidinophenyl)propanoic acid(F4G)
WWVDVKDDLYFVDCG

SEQ ID NO: 18 - protein, 15 aa, synthetic construct
  MOD_RES 12: note = Y represents homo-L-tyrosine(Hty)
WWVDVKDDLYFYDCG

SEQ ID NO: 19 - protein, 15 aa, synthetic construct
  MOD_RES 3: note = L represents (S)-2-Amino-3,3-dimethylbutanoic acid(Tbg)
  MOD_RES 11: note = Y represents (S)-2-Amino-3-(4-phenoxyphenyl)propanoic acid(Yph)
WWLDVKDDLYYVDCG

SEQ ID NO: 20 - protein, 15 aa, synthetic construct
  MOD_RES 3: note = L represents (S)-2-Amino-3,3-dimethylbutanoic acid(Tbg)
  MOD_RES 11: note = Y represents (S)-2-Amino-3-(4-phenoxyphenyl)propanoic acid(Yph)
  MOD_RES 12: note = Y represents homo-L-tyrosine(Hty)
WWLDVKDDLYYYDCG

SEQ ID NO: 21 - protein, 15 aa, synthetic construct
  MOD_RES 1: note = K represents N6-carbamoyl-L-lysine(Hcit)
  MOD_RES 3: note = L represents (S)-2-Amino-3,3-dimethylbutanoic acid(Tbg)
  MOD_RES 12: note = Y represents homo-L-tyrosine(Hty)
KWLDVKDDLYFYDCG

SEQ ID NO: 22 - protein, 15 aa, synthetic construct
  MOD_RES 1: note = A represents (S)-2-Amino-3-(2-aminopyridin-4-yl)propanoic acid(4Py2NH2)
  MOD_RES 3: note = L represents (S)-2-Amino-3,3-dimethylbutanoic acid(Tbg)
  MOD_RES 12: note = Y represents homo-L-tyrosine(Hty)
AWLDVKDDLYFYDCG

SEQ ID NO: 23 - protein, 15 aa, synthetic construct
  MOD_RES 1: note = A represents (S)-2-Amino-3-(6-aminopyridin-3-yl) propanoic acid(3Py6NH2)
  MOD_RES 3: note = L represents (S)-2-Amino-3,3-dimethylbutanoic acid(Tbg)
  MOD_RES 12: note = Y represents homo-L-tyrosine(Hty)
AWLDVKDDLYFYDCG

SEQ ID NO: 24 - protein, 15 aa, synthetic construct
  MOD_RES 1: note = F represents (S)-2-Amino-3-(4-(carboxymethoxy) phenyl) propanoic acid(F4aao)
  MOD_RES 3: note = L represents (S)-2-Amino-3,3-dimethylbutanoic acid(Tbg)
  MOD_RES 12: note = Y represents homo-L-tyrosine(Hty)
FWLDVKDDLYFYDCG

SEQ ID NO: 25 - protein, 15 aa, synthetic construct
  MOD_RES 3: note = G represents (S)-2-Amino-2-cyclohexylacetic acid(Chg)
  MOD_RES 12: note = Y represents homo-L-tyrosine(Hty)
WWGDVKDDLYFYDCG

SEQ ID NO: 26 - protein, 15 aa, synthetic construct
  MOD_RES 3: note = L represents (S)-2-Amino-3,3-dimethylbutanoic acid(Tbg)
  MOD_RES 12: note = Y represents homo-L-tyrosine(Hty)
WWLQVKDDLYFYDCG

SEQ ID NO: 27 - protein, 15 aa, synthetic construct
  MOD_RES 3: note = L represents (S)-2-Amino-3,3-dimethylbutanoic acid(Tbg)
  MOD_RES 5: note = T represents allo-threonine(alT)
  MOD_RES 12: note = Y represents homo-L-tyrosine(Hty)
WWLDTKDDLYFYDCG

SEQ ID NO: 28 - protein, 15 aa, synthetic construct
  MOD_RES 3: note = L represents (S)-2-Amino-3,3-dimethylbutanoic acid(Tbg)
  MOD_RES 5: note = G represents (S)-2-Amino-2-cyclohexylacetic acid(Chg)
  MOD_RES 12: note = Y represents homo-L-tyrosine(Hty)
WWLDGKDDLYFYDCG

SEQ ID NO: 29 - protein, 15 aa, synthetic construct
  MOD_RES 3: note = L represents (S)-2-Amino-3,3-dimethylbutanoic acid(Tbg)
  MOD_RES 12: note = Y represents homo-L-tyrosine(Hty)
WWLDVKDDNYFYDCG

SEQ ID NO: 30 - protein, 15 aa, synthetic construct
  MOD_RES 3: note = L represents (S)-2-Amino-3,3-dimethylbutanoic acid(Tbg)
  MOD_RES 11: note = F represents (S)-2-Amino-3-(4-chlorophenyl)propanoic acid(F4C)
  MOD_RES 12: note = Y represents homo-L-tyrosine(Hty)
WWLDVKDDLYFYDCG

SEQ ID NO: 31 - protein, 15 aa, synthetic construct
  MOD_RES 3: note = L represents (S)-2-Amino-3,3-dimethylbutanoic acid(Tbg)
  MOD_RES 12: note = G represents (S)-2-Amino-2-cyclohexylacetic acid(Chg)
WWLDVKDDLYFGDCG

SEQ ID NO: 32 - protein, 15 aa, synthetic construct
  MOD_RES 3: note = L represents (S)-2-Amino-3,3-dimethylbutanoic acid(Tbg)
  MOD_RES 12: note = X represents (S)-2-Amino-4-(pyridin-4-yl)butanoic acid(H4Py)
WWLDVKDDLYFXDCG

SEQ ID NO: 33 - protein, 15 aa, synthetic construct
  MOD_RES 3: note = L represents (S)-2-Amino-3,3-dimethylbutanoic acid(Tbg)
  MOD_RES 12: note = Y represents homo-L-tyrosine(Hty)
WWLDVKDDLYFYSCG

SEQ ID NO: 34 - protein, 15 aa, synthetic construct
  MOD_RES 3: note = L represents (S)-2-Amino-3,3-dimethylbutanoic acid(Tbg)
  MOD_RES 12: note = Y represents homo-L-tyrosine(Hty)
WWLDVKDDLYFYFCG

SEQ ID NO: 35 - protein, 15 aa, synthetic construct
  MOD_RES 3: note = L represents (S)-2-Amino-3,3-dimethylbutanoic acid(Tbg)
  MOD_RES 12: note = Y represents homo-L-tyrosine(Hty)
  MOD_RES 13: note = F represents (S)-2-Amino-3-(4-(carboxymethoxy) phenyl) propanoic acid(F4aao)
WWLDVKDDLYFYFCG

SEQ ID NO: 36 - protein, 15 aa, synthetic construct
  MOD_RES 3: note = L represents (S)-2-Amino-3,3-dimethylbutanoic acid(Tbg)
  MOD_RES 6: note = X represents (S)-2-Aminoheptanoic acid(Ahp)
  MOD_RES 12: note = Y represents homo-L-tyrosine(Hty)
WWLDVXDDLYFYDCG

SEQ ID NO: 37 - protein, 15 aa, synthetic construct
  MOD_RES 12: note = Y represents homo-L-tyrosine(Hty)
WWVDVKGVNYFYDCG

SEQ ID NO: 38 - protein, 15 aa, synthetic construct
  MOD_RES 4: note = M represents (S)-2-Amino-4-(methylsulfonyl)butanoic acid(MetO2)
  MOD_RES 12: note = Y represents homo-L-tyrosine(Hty)
WWVMVKDDLYFYDCG

SEQ ID NO: 39 - protein, 15 aa, synthetic construct
  MOD_RES 11: note = Y represents (S)-2-Amino-3-(4-phenoxyphenyl)propanoic acid(Yph)
  MOD_RES 13: note = K represents N6-carbamimidoyl-L-lysine(Har)
WWVDVKDDLYYVKCG

SEQ ID NO: 40 - protein, 15 aa, synthetic construct
  MOD_RES 3: note = Y represents homo-L-tyrosine(Hty)
  MOD_RES 11: note = F represents (S)-2-Amino-3-(4-guanidinophenyl)propanoic acid(F4G)
WWYDVKDDLYFVDCG

SEQ ID NO: 41 - protein, 15 aa, synthetic construct
  MOD_RES 11: note = F represents (S)-2-Amino-3-(4-guanidinophenyl)propanoic acid(F4G)
  MOD_RES 12: note = Y represents homo-L-tyrosine(Hty)
  MOD_RES 13: note = P represents hydroxyproline(Hyp)
WWVDVKDDLYFYPCG

SEQ ID NO: 42 - protein, 15 aa, synthetic construct
  MOD_RES 3: note = L represents (S)-2-Amino-3,3-dimethylbutanoic acid(Tbg)
  MOD_RES 11: note = F represents (S)-2-Amino-3-(4-guanidinophenyl)propanoic acid(F4G)
WWLDVKDDLYFVDCG

SEQ ID NO: 43 - protein, 15 aa, synthetic construct
  MOD_RES 3: note = L represents (S)-2-Amino-3,3-dimethylbutanoic acid(Tbg)
  MOD_RES 12: note = Y represents homo-L-tyrosine(Hty)
WWLDVKDDLYFYDCG

SEQ ID NO: 44 - protein, 15 aa, synthetic construct
  MOD_RES 3: note = L represents (S)-2-Amino-3,3-dimethylbutanoic acid(Tbg)
  MOD_RES 11: note = F represents (S)-2-Amino-3-(4-guanidinophenyl)propanoic acid(F4G)
  MOD_RES 12: note = Y represents homo-L-tyrosine(Hty)
WWLDVKDDLYFYDCG

SEQ ID NO: 45 - protein, 15 aa, synthetic construct
  MOD_RES 1: note = W represents (S)-2-Amino-3-(1H-pyrrolo[2,3-b]pyridin-3-yl)propanoic acid(W7N)
  MOD_RES 3: note = L represents (S)-2-Amino-3,3-dimethylbutanoic acid(Tbg)
  MOD_RES 12: note = Y represents homo-L-tyrosine(Hty)
WWLDVKDDLYFYDCG

SEQ ID NO: 46 - protein, 15 aa, synthetic construct
  MOD_RES 3: note = L represents (S)-2-Amino-3,3-dimethylbutanoic acid(Tbg)
  MOD_RES 12: note = Y represents homo-L-tyrosine(Hty)
WWLDVKNDLYFYDCG

SEQ ID NO: 47 - protein, 15 aa, synthetic construct
  MOD_RES 3: note = L represents (S)-2-Amino-3,3-dimethylbutanoic acid(Tbg)
  MOD_RES 9: note = A represents (S)-2-Amino-4,4-dimethylpentanoic acid(Atb)
  MOD_RES 12: note = Y represents homo-L-tyrosine(Hty)
WWLDVKDDAYFYDCG

SEQ ID NO: 48 - protein, 15 aa, synthetic construct
  MOD_RES 3: note = L represents (S)-2-Amino-3,3-dimethylbutanoic acid(Tbg)
  MOD_RES 9: note = A represents (S)-2-Amino-4,4-dimethylpentanoic acid(Atb)
  MOD_RES 11: note = F represents (S)-2-Amino-3-(4-guanidinophenyl)propanoic acid(F4G)
  MOD_RES 12: note = Y represents homo-L-tyrosine(Hty)
WWLDVKDDAYFYDCG

SEQ ID NO: 49 - protein, 15 aa, synthetic construct
  MOD_RES 3: note = L represents (S)-2-Amino-3,3-dimethylbutanoic acid(Tbg)
  MOD_RES 9: note = A represents (S)-2-Amino-4,4-dimethylpentanoic acid(Atb)
  MOD_RES 11: note = F represents (S)-2-Amino-3-(4-guanidinophenyl)propanoic acid(F4G)
  MOD_RES 12: note = Y represents homo-L-tyrosine(Hty)
  MOD_RES 13: note = P represents hydroxyproline(Hyp)
WWLDVKDDAYFYPCG

SEQ ID NO: 50 - protein, 15 aa, synthetic construct
  MOD_RES 3: note = Y represents homo-L-tyrosine(Hty)
  MOD_RES 9: note = A represents (S)-2-Amino-4,4-dimethylpentanoic acid(Atb)
  MOD_RES 11: note = F represents (S)-2-Amino-3-(4-guanidinophenyl)propanoic acid(F4G)
WWYDVKDDAYFVDCG

SEQ ID NO: 51 - protein, 15 aa, synthetic construct
  MOD_RES 3: note = Y represents homo-L-tyrosine(Hty)
  MOD_RES 9: note = A represents (S)-2-Amino-4,4-dimethylpentanoic acid(Atb)
  MOD_RES 11: note = F represents (S)-2-Amino-3-(4-guanidinophenyl)propanoic acid(F4G)
  MOD_RES 12: note = Y represents homo-L-tyrosine(Hty)
WWYDVKDDAYFYDCG